European Patent Application EP 4 501 966 A1, published February 5, 2025. Title: ANTIBODY SPECIFICALLY BINDING TO HUMAN DR3 AND USE THEREOF. Applicant: SELECXINE INC. Application EP. The sequence listing filed with the application follows.

SEQUENCE LISTING (84 sequences)

SEQ ID NO: 1 - protein, 10 aa, synthetic construct
GYTFTSYGIS

SEQ ID NO: 2 - protein, 17 aa, synthetic construct
WISAYNGNTNYAQKLQG

SEQ ID NO: 3 - protein, 11 aa, synthetic construct
ASGPDYGMLDY

SEQ ID NO: 4 - protein, 9 aa, synthetic construct
QASQDISNY

SEQ ID NO: 5 - protein, 7 aa, synthetic construct
DASNLET

SEQ ID NO: 6 - protein, 9 aa, synthetic construct
QQYDNLPLT

SEQ ID NO: 7 - protein, 12 aa, synthetic construct
GGSISSSSYYWG

SEQ ID NO: 8 - protein, 16 aa, synthetic construct
SIYYSGSTYYNPSLKS

SEQ ID NO: 9 - protein, 10 aa, synthetic construct
ARQVSGPLDY

SEQ ID NO: 10 - protein, 11 aa, synthetic construct
RASQGIRNDLG

SEQ ID NO: 11 - protein, 7 aa, synthetic construct
AASSLQS

SEQ ID NO: 12 - protein, 9 aa, synthetic construct
LQDYNYPRT

SEQ ID NO: 13 - protein, 10 aa, synthetic construct
GFTFSDYYMS

SEQ ID NO: 14 - protein, 17 aa, synthetic construct
YISSSSSYTNYADSVKG

SEQ ID NO: 15 - protein, 14 aa, synthetic construct
ASNVDTAMVGAFDI

SEQ ID NO: 16 - protein, 11 aa, synthetic construct
RASQHISNWLA

SEQ ID NO: 17 - protein, 7 aa, synthetic construct
TASNLQS

SEQ ID NO: 18 - protein, 9 aa, synthetic construct
QQADSFPLT

SEQ ID NO: 19 - protein, 10 aa, synthetic construct
GFTFSSYSMN

SEQ ID NO: 20 - protein, 17 aa, synthetic construct
YISSSSSTIYYADSVKG

SEQ ID NO: 21 - protein, 18 aa, synthetic construct
ARWDGYCSGGSCYSGMDY

SEQ ID NO: 22 - protein, 11 aa, synthetic construct
QASQDISNYLN

SEQ ID NO: 23 - protein, 7 aa, synthetic construct
DASNLET

SEQ ID NO: 24 - protein, 9 aa, synthetic construct
QQYDNLPLT

SEQ ID NO: 25 - protein, 10 aa, synthetic construct
GFTFSSYSMN

SEQ ID NO: 26 - protein, 17 aa, synthetic construct
YISSSSSTIYYADSVKG

SEQ ID NO: 27 - protein, 18 aa, synthetic construct
ARWDGYCSGGSCYSGMDY

SEQ ID NO: 28 - protein, 11 aa, synthetic construct
QASQDISNYLN

SEQ ID NO: 29 - protein, 7 aa, synthetic construct
DASNLET

SEQ ID NO: 30 - protein, 9 aa, synthetic construct
QQYDNLPLT

SEQ ID NO: 31 - DNA, 30 bp, synthetic construct
  source 1..30: mol_type = other DNA
ggttacacctttaccagctatggtatcagc

SEQ ID NO: 32 - DNA, 51 bp, synthetic construct
  source 1..51: mol_type = other DNA
tggatcagcgcttacaatggtaacacaaactatgcacagaagctccagggc

SEQ ID NO: 33 - DNA, 33 bp, synthetic construct
  source 1..33: mol_type = other DNA
gcgagtggccccgactacggcatgcttgactac

SEQ ID NO: 34 - DNA, 27 bp, synthetic construct
  source 1..27: mol_type = other DNA
caggcgagtcaggacattagcaactac

SEQ ID NO: 35 - DNA, 21 bp, synthetic construct
  source 1..21: mol_type = other DNA
gatgcatccaatttggaaaca

SEQ ID NO: 36 - DNA, 27 bp, synthetic construct
  source 1..27: mol_type = other DNA
caacagtatgataatctccccctcact

SEQ ID NO: 37 - DNA, 36 bp, synthetic construct
  source 1..36: mol_type = other DNA
ggtggctccatcagcagtagtagttactactggggc

SEQ ID NO: 38 - DNA, 48 bp, synthetic construct
  source 1..48: mol_type = other DNA
agtatctattatagtgggagcacctactacaacccgtccctcaagagt

SEQ ID NO: 39 - DNA, 30 bp, synthetic construct
  source 1..30: mol_type = other DNA
gcgaggcaagtttcggggccccttgactac

SEQ ID NO: 40 - DNA, 33 bp, synthetic construct
  source 1..33: mol_type = other DNA
cgggcaagtcagggcattagaaatgatttaggc

SEQ ID NO: 41 - DNA, 21 bp, synthetic construct
  source 1..21: mol_type = other DNA
gctgcatccagtttacaaagt

SEQ ID NO: 42 - DNA, 27 bp, synthetic construct
  source 1..27: mol_type = other DNA
ctacaagattacaattaccctcggacg

SEQ ID NO: 43 - DNA, 30 bp, synthetic construct
  source 1..30: mol_type = other DNA
ggattcaccttcagtgactactacatgagc

SEQ ID NO: 44 - DNA, 51 bp, synthetic construct
  source 1..51: mol_type = other DNA
tacattagtagtagtagtagttacacaaactacgcagactctgtgaagggc

SEQ ID NO: 45 - DNA, 42 bp, synthetic construct
  source 1..42: mol_type = other DNA
gcgagtaacgtggatacagctatggttggggcttttgatatc

SEQ ID NO: 46 - DNA, 33 bp, synthetic construct
  source 1..33: mol_type = other DNA
cgggcgagtcaacatattagcaactggttagcc

SEQ ID NO: 47 - DNA, 21 bp, synthetic construct
  source 1..21: mol_type = other DNA
actgcatccaatttgcaaagt

SEQ ID NO: 48 - DNA, 27 bp, synthetic construct
  source 1..27: mol_type = other DNA
caacaggctgacagtttcccgctcact

SEQ ID NO: 49 - DNA, 30 bp, synthetic construct
  source 1..30: mol_type = other DNA
ggattcaccttcagtagctatagcatgaac

SEQ ID NO: 50 - DNA, 51 bp, synthetic construct
  source 1..51: mol_type = other DNA
tacattagtagtagtagtagcaccatatactacgcagactctgtgaagggc

SEQ ID NO: 51 - DNA, 51 bp, synthetic construct; identical to SEQ ID NO: 50
  source 1..51: mol_type = other DNA

SEQ ID NO: 52 - DNA, 33 bp, synthetic construct
  source 1..33: mol_type = other DNA
caggcgagtcaggacattagcaactatttaaat

SEQ ID NO: 53 - DNA, 21 bp, synthetic construct
  source 1..21: mol_type = other DNA
gatgcatccaatttggaaaca

SEQ ID NO: 54 - DNA, 27 bp, synthetic construct
  source 1..27: mol_type = other DNA
caacagtatgataatctccccctcact

SEQ ID NO: 55 - DNA, 30 bp, synthetic construct; identical to SEQ ID NO: 49
  source 1..30: mol_type = other DNA

SEQ ID NO: 56 - DNA, 51 bp, synthetic construct; identical to SEQ ID NO: 50
  source 1..51: mol_type = other DNA

SEQ ID NO: 57 - DNA, 54 bp, synthetic construct
  source 1..54: mol_type = other DNA
gcgagatgggatggatattgtagtggtggtagctgctactccgggatggactac

SEQ ID NO: 58 - DNA, 33 bp, synthetic construct; identical to SEQ ID NO: 52
  source 1..33: mol_type = other DNA

SEQ ID NO: 59 - DNA, 21 bp, synthetic construct
  source 1..21: mol_type = other DNA
gatgcatccaatttggaaaca

SEQ ID NO: 60 - DNA, 27 bp, synthetic construct
  source 1..27: mol_type = other DNA
caacagtatgataatctccctctcact

SEQ ID NO: 61 - DNA, 351 bp, synthetic construct
  source 1..351: mol_type = other DNA
caggtgcagctggtgcagtctggagctgaggtgaagaagcctggggcctcagtgaaggtctcctgcaaggcttctggttacacctttaccagctatggtatcagctgggtgcgacaggcccctggacaagggcttgagtggatgggatggatcagcgcttacaatggtaacacaaactatgcacagaagctccagggcagagtcaccatgaccacagacacatccacgagcacagcctacatggagctgaggagcctgagatctgacgacacggccgtgtattactgtgcgagtggccccgactacggcatgcttgactactggggccagggcaccctggtcaccgtctcc

SEQ ID NO: 62 - DNA, 321 bp, synthetic construct
  source 1..321: mol_type = other DNA
gaaattgtgatgacgcagtctccatcctccctgcctgcatctgtaggagacagagtcaccatcacttgccaggcgagtcaggacattagcaactacttaaattggtatcagcagaaaccagggaaagcccctaagctcctgatctacgatgcatccaatttggaaacaggggtcccatcaaggttcagtggaagtggatctgggacagattttactttcaccatcagcagcccgcagcctgaagatattgcaacatattactgtcaacagtatgataatctccccctcactttcggcggagggaccaaggtggagatcaaa

SEQ ID NO: 63 - protein, 117 aa, synthetic construct
QVQLVQSGAEVKKPGASVKVSCKASGYTFTSYGISWVRQAPGQGLEWMGWISAYNGNTNYAQKLQGRVTMTTDTSTSTAYMELRSLRSDDTAVYYCASGPDYGMLDYWGQGTLVTVS

SEQ ID NO: 64 - protein, 107 aa, synthetic construct
EIVMTQSPSSLPASVGDRVTITCQASQDISNYLNWYQQKPGKAPKLLIYDASNLETGVPSRFSGSGSGTDFTFTISSPQPEDIATYYCQQYDNLPLTFGGGTKVEIK

SEQ ID NO: 65 - DNA, 351 bp, synthetic construct
  source 1..351: mol_type = other DNA
caggtgcagctgcagcagtcgggcccaggactggtgaagccttcggagaccctgtccctcacctgcactgtctctggtggctccatcagcagtagtagttactactggggctggatccgccagcccccagggaaggggctggagtggattgggagtatctattatagtgggagcacctactacaacccgtccctcaagagtcgagtcaccatatccgtagacacgtccaagaaccagttctccctgaagctgagctctgtgaccgccgcagacacggctgtgtattactgtgcgaggcaagtttcggggccccttgactactggggccaggggaccctggtcaccgtctcc

SEQ ID NO: 66 - DNA, 321 bp, synthetic construct
  source 1..321: mol_type = other DNA
gacatcgtgatgacccagtctccatcctccctgtctgcatctgtaggagacagagtcaccatcacttgccgggcaagtcagggcattagaaatgatttaggctggtatcagcagaaaccagggaaagcccctaagctcctgatctatgctgcatccagtttacaaagtggggtcccatcaaggttcagcggcagtggatctggcacagatttcactctcaccatcagcagcctgcagcctgaagattttgcaacttattactgtctacaagattacaattaccctcggacgttcggccaagggaccaaggtggaaatcaaa

SEQ ID NO: 67 - protein, 117 aa, synthetic construct
QVQLQQSGPGLVKPSETLSLTCTVSGGSISSSSYYWGWIRQPPGKGLEWIGSIYYSGSTYYNPSLKSRVTISVDTSKNQFSLKLSSVTAADTAVYYCARQVSGPLDYWGQGTLVTVS

SEQ ID NO: 68 - protein, 107 aa, synthetic construct
DIVMTQSPSSLSASVGDRVTITCRASQGIRNDLGWYQQKPGKAPKLLIYAASSLQSGVPSRFSGSGSGTDFTLTISSLQPEDFATYYCLQDYNYPRTFGQGTKVEIK

SEQ ID NO: 69 - DNA, 360 bp, synthetic construct
  source 1..360: mol_type = other DNA
gaggtgcagctggtggagtctgggggaggcttggtcaagcctggagggtccctgagactctcctgtgcagcctctggattcaccttcagtgactactacatgagctggatccgccaggctccagggaaggggctggagtgggtttcatacattagtagtagtagtagttacacaaactacgcagactctgtgaagggccgattcaccatctccagagacaacgccaagaactcactgtatctgcaaatgaacagcctgagagccgaggacacggccgtgtattactgtgcgagtaacgtggatacagctatggttggggcttttgatatctggggccaaggaaccctggtcaccgtctcc

SEQ ID NO: 70 - DNA, 321 bp, synthetic construct
  source 1..321: mol_type = other DNA
gacatcgagatgacccagtctccttcttccgtgtctgcatctgtaggagacacagtcaccatcacctgccgggcgagtcaacatattagcaactggttagcctggtatcagcagaaaccagggcaagcccctaagttcctgatctatactgcatccaatttgcaaagtggggtcccatcaagattcagcggcagtggatatgggacagatttcactctcaccatcagcggcctgcagcctgaagattttgcgacttactattgtcaacaggctgacagtttcccgctcactttcggcggagggaccaaggtggatatcaaa

SEQ ID NO: 71 - protein, 120 aa, synthetic construct
EVQLVESGGGLVKPGGSLRLSCAASGFTFSDYYMSWIRQAPGKGLEWVSYISSSSSYTNYADSVKGRFTISRDNAKNSLYLQMNSLRAEDTAVYYCASNVDTAMVGAFDIWGQGTLVTVS

SEQ ID NO: 72 - protein, 107 aa, synthetic construct
DIEMTQSPSSVSASVGDTVTITCRASQHISNWLAWYQQKPGQAPKFLIYTASNLQSGVPSRFSGSGYGTDFTLTISGLQPEDFATYYCQQADSFPLTFGGGTKVDIK

SEQ ID NO: 73 - DNA, 372 bp, synthetic construct
  source 1..372: mol_type = other DNA
caggtgcagctggtgcagtctgggggaggcttggtacagcctggggggtccctgagactctcctgtgcagcctctggattcaccttcagtagctatagcatgaactgggtccgccaggctccagggaaggggctggagtgggtttcatacattagtagtagtagtagcaccatatactacgcagactctgtgaagggccgattcaccatctccagagacaacgccaagaactcactgtatctgcaaatgaacagcctgagagccgaggacacggctgtgtattactgtgcgagatgggatggatattgtagtggtggtagctgctactccgggatggactactggggccagggcaccctggtcaccgtctcc

SEQ ID NO: 74 - DNA, 321 bp, synthetic construct
  source 1..321: mol_type = other DNA
gacatcgagatgacccagtctccatcctccctgtctgcatctgtaggagacagagtcaccatcacttgccaggcgagtcaggacattagcaactatttaaattggtatcagcagaaaccagggaaagcccctaagctcctgatctacgatgcatccaatttggaaacaggggtcccatcaaggttcagtggaagtggatctgggacagattttactttcaccatcagcagcctgcagcctgaagatattgcaacatattactgtcaacagtatgataatctccccctcactttcggcggagggaccaaggtggagatcaaa

SEQ ID NO: 75 - protein, 124 aa, synthetic construct
QVQLVQSGGGLVQPGGSLRLSCAASGFTFSSYSMNWVRQAPGKGLEWVSYISSSSSTIYYADSVKGRFTISRDNAKNSLYLQMNSLRAEDTAVYYCARWDGYCSGGSCYSGMDYWGQGTLVTVS

SEQ ID NO: 76 - protein, 107 aa, synthetic construct
DIEMTQSPSSLSASVGDRVTITCQASQDISNYLNWYQQKPGKAPKLLIYDASNLETGVPSRFSGSGSGTDFTFTISSLQPEDIATYYCQQYDNLPLTFGGGTKVEIK

SEQ ID NO: 77 - DNA, 372 bp, synthetic construct; identical to SEQ ID NO: 73
  source 1..372: mol_type = other DNA

SEQ ID NO: 78 - DNA, 321 bp, synthetic construct
  source 1..321: mol_type = other DNA
gacatcgagatgacccagtctccatcctccctgtctgcatctgtaggagacaaagtcaccatcacttgccaggcgagtcaggacattagcaactatttaaattggtatcagcagaaaccagggaaagcccctaagctcctgatctacgatgcatccaatttggaaacaggggtcccatcaaggttcagtggaagtggatctgggacagattctactttcaccatcagcagcctgcagcctgaagatattgcaacatattactgtcaacagtatgataatctccctctcactttcggcggagggaccaaggtggagatcaaa

SEQ ID NO: 79 - protein, 124 aa, synthetic construct; identical to SEQ ID NO: 75

SEQ ID NO: 80 - protein, 107 aa, synthetic construct
DIEMTQSPSSLSASVGDKVTITCQASQDISNYLNWYQQKPGKAPKLLIYDASNLETGVPSRFSGSGSGTDSTFTISSLQPEDIATYYCQQYDNLPLTFGGGTKVEIK

SEQ ID NO: 81 - DNA, 1347 bp, synthetic construct
  source 1..1347: mol_type = other DNA
gaggtgcagctggtggagagcggggggggactggtgaagccagggggaagcctgagactgagctgtgccgcaagcgggttcacatttagtgactattatatgagttggatcagacaggcacccggcaaaggactggagtgggtgagctacatcagcagcagtagcagctacaccaactacgccgacagtgtgaagggcagattcaccatcagcagagacaacgccaagaacagcctgtacctgcagatgaacagcctgagagccgaggacaccgccgtgtactactgcgcaagcaacgtggacaccgctatggtgggggccttcgacatctggggacaaggaacactcgtgaccgtgagcagcgctagcaccaagggcccatcggtcttccccctggcgccctgctccaggagcacctccgagagcacagccgccctgggctgcctggtcaaggactacttccccgaaccggtgacggtgtcgtggaactcaggcgccctgaccagcggcgtgcacaccttcccggctgtcctacagtcctcaggactctactccctcagcagcgtggtgaccgtgccctccagcagcttgggcacgaagacctacacctgcaacgtagatcacaagcccagcaacaccaaggtggacaagagagttgagtccaaatatggtcccccatgcccaccatgcccagcacctgagttcctggggggaccatcagtcttcctgttccccccaaaacccaaggacactctcatgatctcccggacccctgaggtcacgtgcgtggtggtggacgtgagccaggaagaccccgaggtccagttcaactggtacgtggatggcgtggaggtgcataatgccaagacaaagccgcgggaggagcagttcaacagcacgtaccgtgtggtcagcgtcctcaccgtcctgcaccaggactggctgaacggcaaggagtacaagtgcaaggtctccaacaaaggcctcccgtcctccatcgagaaaaccatctccaaagccaaagggcagccccgagagccacaggtgtacaccctgcccccatcccaggaggagatgaccaagaaccaggtcagcctgacctgcctggtcaaaggcttctaccccagcgacatcgccgtggagtgggagagcaatgggcagccggagaacaactacaagaccacgcctcccgtgctggactccgacggctccttcttcctctacagcaggctaaccgtggacaagagcaggtggcaggaggggaatgtcttctcatgctccgtgatgcatgaggctctgcacaaccactacacacagaagagcctctccctgtctctgggtaaatga

SEQ ID NO: 82 - DNA, 645 bp, synthetic construct
  source 1..645: mol_type = other DNA
gacattgaaatgacccagagccccagcagcgtgagcgccagcgtgggagacaccgtgaccatcacctgcagagcaagccaacacataagcaactggctggcctggtaccagcagaaacccggacaggcccccaaattcctcatctacaccgcaagtaacctgcaaagcggcgtgcccagcagattcagcggcagcggctacggcaccgacttcaccctcaccatcagcggactgcaacccgaggacttcgccacctactactgccaacaagccgacagcttccccctgaccttcggcggaggcaccaaggtggatatcaagcgtacggtggctgcaccatctgtcttcatcttcccgccatctgatgagcagttgaaatctggaactgcctctgttgtgtgcctgctgaataacttctatcccagagaggccaaagtacagtggaaggtggataacgccctccaatcgggtaactcccaggagagtgtcacagagcaggacagcaaggacagcacctacagcctcagcagcaccctgacgctgagcaaagcagactacgagaaacacaaagtctacgcctgcgaagtcacccatcagggcctgagttcgcccgtcacaaagagcttcaacaggggagagtgttga

SEQ ID NO: 83 - protein, 448 aa, synthetic construct
EVQLVESGGGLVKPGGSLRLSCAASGFTFSDYYMSWIRQAPGKGLEWVSYISSSSSYTNYADSVKGRFTISRDNAKNSLYLQMNSLRAEDTAVYYCASNVDTAMVGAFDIWGQGTLVTVSSASTKGPSVFPLAPCSRSTSESTAALGCLVKDYFPEPVTVSWNSGALTSGVHTFPAVLQSSGLYSLSSVVTVPSSSLGTKTYTCNVDHKPSNTKVDKRVESKYGPPCPPCPAPEFLGGPSVFLFPPKPKDTLMISRTPEVTCVVVDVSQEDPEVQFNWYVDGVEVHNAKTKPREEQFNSTYRVVSVLTVLHQDWLNGKEYKCKVSNKGLPSSIEKTISKAKGQPREPQVYTLPPSQEEMTKNQVSLTCLVKGFYPSDIAVEWESNGQPENNYKTTPPVLDSDGSFFLYSRLTVDKSRWQEGNVFSCSVMHEALHNHYTQKSLSLSLGK

SEQ ID NO: 84 - protein, 214 aa, synthetic construct
DIEMTQSPSSVSASVGDTVTITCRASQHISNWLAWYQQKPGQAPKFLIYTASNLQSGVPSRFSGSGYGTDFTLTISGLQPEDFATYYCQQADSFPLTFGGGTKVDIKRTVAAPSVFIFPPSDEQLKSGTASVVCLLNNFYPREAKVQWKVDNALQSGNSQESVTEQDSKDSTYSLSSTLTLSKADYEKHKVYACEVTHQGLSSPVTKSFNRGEC